European Patent Application EP 4 209 579 A1, published July 12, 2023. Title: Bifidobacteria for suppressing atrogene expression. Applicant: NISSIN FOODS HOLDINGS CO., LTD. The sequence listing filed with the application follows.

SEQUENCE LISTING (4 sequences)

SEQ ID NO: 1 - DNA, 20 bp, Artificial Sequence
  A primer for gene expression measurement by RT-PCR
tgggggagccaccttcctct

SEQ ID NO: 2 - DNA, 25 bp, Artificial Sequence
  A primer for gene expression measurement by RT-PCR
atgttctcaaagccctgctctgtct

SEQ ID NO: 3 - DNA, 24 bp, Artificial Sequence
  A primer for gene expression measurement by RT-PCR
ggaaactctgcattctcgcttcct

SEQ ID NO: 4 - DNA, 23 bp, Artificial Sequence
  A primer for gene expression measurement by RT-PCR
ccaggactcgtttgtacccgttg